European Patent Application EP 4 772 610 A1, published July 8, 2026. Title: 락티플란티바실루스 플란타룸 균주 및 이를 포함하는 대사질환의 예방 또는 치료용 조성물. Applicant: 주식회사 지아이바이옴. Application KR. The sequence listing filed with the application follows.

SEQUENCE LISTING (2 sequences)

SEQ ID NO: 1 - DNA, 1426 bp, Lactobacillus plantarum
  source 1..1426: mol_type = genomic DNA
tcgaacgaactctggtattgattggtgcttgcatcatgatttacatttgagtgagtggcgaactggtgagtaacacgtgggaaacctgcccagaagcgggggataacacctggaaacagatgctaataccgcataacaacttggaccgcatggtccgagcttgaaagatggcttcggctatcacttttggatggtcccgcggcgtattagctagatggtggggtaacggctcaccatggcaatgatacgtagccgacctgagagggtaatcggccacattgggactgagacacggcccaaactcctacgggaggcagcagtagggaatcttccacaatggacgaaagtctgatggagcaacgccgcgtgagtgaagaagggtttcggctcgtaaaactctgttgttaaagaagaacatatctgagagtaactgttcaggtattgacggtatttaaccagaaagccacggctaactacgtgccagcagccgcggtaatacgtaggtggcaagcgttgtccggatttattgggcgtaaagcgagcgcaggcggttttttaagtctgatgtgaaagccttcggctcaaccgaagaagtgcatcggaaactgggaaacttgagtgcagaagaggacagtggaactccatgtgtagcggtgaaatgcgtagatatatggaagaacaccagtggcgaaggcggctgtctggtctgtaactgacgctgaggctcgaaagtatgggtagcaaacaggattagataccctggtagtccataccgtaaacgatgaatgctaagtgttggagggtttccgcccttcagtgctgcagctaacgcattaagcattccgcctggggagtacggccgcaaggctgaaactcaaaggaattgacgggggcccgcacaagcggtggagcatgtggtttaattcgaagctacgcgaagaaccttaccaggtcttgacatactatgcaaatctaagagattagacgttcccttcggggacatggatacaggtggtgcatggttgtcgtcagctcgtgtcgtgagatgttgggttaagtcccgcaacgagcgcaacccttattatcagttgccagcattaagttgggcactctggtgagactgccggtgacaaaccggaggaaggtggggatgacgtcaaatcatcatgccccttatgacctgggctacacacgtgctacaatggatggtacaacgagttgcgaactcgcgagagtaagctaatctcttaaagccattctcagttcggattgtaggctgcaactcgcctacatgaagtcggaatcgctagtaatcgcggatcagcatgccgcggtgaatacgttcccgggccttgtacacaccgcccgtcacaccatgagagtttgtaacacccaaagtcggtggggtaacctttttagaactcag

SEQ ID NO: 2 - DNA, 684 bp, Lactobacillus plantarum
  source 1..684: mol_type = genomic DNA
ttcggtaaaggggcgattatgcggatgggtgacgctgcccagacgactatttcaacgatttcaagtggatcgttggccttagatgacgcgttgggtgtcggcggctacccacgtggtcggatcgtggaaatctacggtcctgaaagttcaggtaaaacgaccgtggcactacatgcggttgctgaagttcaaaagcagggtggtacggcggcctatatcgatgctgaaaacgcactagaccccgtttatgcggaacacctaggggtcaacattgatgacctgttactttcgcaaccagatactggtgaacaagggcttgaaattgcagatgccttagtttccagtggtgcggtcgatattttagttgttgactcggtggcggccttagtgccacgtgccgaaattgaaggtgaaatgggtgacgcacacgttgggttacaagcgcggctgatgtcacaagcgctccggaagttatcagggacattgaacaaaaccaagacaatcgcgttatttatcaatcaaattcgtgaaaaagttggtgtgatgtttggtaatcctgaaacgactcctggtggtcgggccttgaaattttacgccacgattcgtttggaagtacggcgggcagaacagatcaaggaaggaaccaatattattggtaaccgtgtccggatcaaagtcgttaag